European Patent Specification EP 3 442 992 B1, published April 10, 2024. Title: METHODS FOR IDENTIFYING MODULATORS OF GPR92. Applicant: MARS, INCORPORATED. The sequence listing filed with the application follows.

SEQUENCE LISTING (6 sequences)

SEQ ID NO: 1 - DNA, 1122 bp, Felis catus
atgttgcccaactctaccaacagttctgttccccctgccaacggttctgttcccccgtgccccgactaccggcccacccaccgcctgcacatggtggcctacagcctggtgctggccgcagggctccccctcaacgcgctggccctctgggtcttcctgcgcgcgctgcgagtgcactccgtcgtgagcgtgtacatgtgcaacctggcggccagcgacctgctcttcaccctctcgctgcccgtgcgcatctcctactacgccctgcactactggcccttctccgacctcctgtgccagacggcgggcgccatcttccagacgaacatgtacggcagctgcatcttcctgactctcatcaacgtggaccgctacgcggccatcgtgcacccgctgcggctgcgccacctgcggcggccccgcgtggcgcggctgctctgcctgggagtgtgggcgctcatcctcgtgttcgctgtgcccaccgtcctggtgcacaggccctcgtcctgcagctacggcggcggccaggtgcgcctgtgcttcgagagcttcggcgacaggctgtggaagggcgggctgctgccgctcgtgctgctggccgaggcgctgggcttcctgctgcccctggtggcggtgctctactcgtcgggccgggtcttctggaccctggcgcggcccgacgccacgcagagccagcggcggcggaagaccgtgcgcctcctgctggccaacctcgtcatcttcctgctgtgcttcgtgccctacaacgccacgctggcggtgtacgggctgctgcggggcaacctggtggcggcgaacagcaaggtctgcgatcgggtgcgcggggtgctgatggtgatggtgctgttggccggcgccaactgcgtgctagaccctctggtgtattacttcagcgccgagggtttccgcaacaccctgcgaggcctgggcactccgaaccgcgccaggaccttggccaccaacggggctcagggggcgctcgccgaacagcccactgagaccacttacatcaccaccccggctaccgccgaacaggggctgctcaggccctccaacgtggggacacccttaacccagctccccgaggactcggccctctga

SEQ ID NO: 2 - DNA, 1101 bp, Canis familiaris
atgctgaccgcctcggccaacagctccgtccccccatgccccgactaccgggtcacccaccgcctgcacatggtggcctacagcctggtgctggccgcggggctccccctcaacgcgctggccctctgggtcttcctgcgcgcgctgcgcgtgcactccgtggtcagcgtgtacatgtgcaacctggcggccagcgacctgctcttcacgctctcgctgcccgtgcgcatctcctactacgccctgcaccactggcccttctccgacctcctgtgtcagacggccggcgccgtcttccagaccaacatgtacggcagctgcatcttcctgaccctcattaacgtggaccgctacgcggccatcgtgcacccactgcggctgcgccacctgcggcggccccgcgtggcgcggctgctgtgcctgggcgtgtgggcgctcatcctggtgttcgccgtgcccaccgtcctggtgcaccggccctcgccctgcagctacgacggcggccgggcgcggctgtgcttcgagagcttcggcgacaagctgtggaagggcgggctgctgccgctcgtgctgctggccgaggcgctgggcttcctgctgccgctcgcggccatgctctactcgtcgggccgggtcttctggaccctggcgcggcccgacgccacgcggagccggcggcggcggaagaccgtgcgcctcctgctggccaacctcgtcatcttcctgctgtgcttcgtgccctacaacgccacgctggccgtctacgggctgctgcggggcaacctggtggcggccggcagcgaggccagcgaccgcgtgcgccaggtgctcatggtgatggtgctgctggccagcgccaactgcgtgctggacccgctggtgtactacttcagcgccgagggcttccgcaacaccctgcgcggcctgggcacttggcaccgtgccaggaccttggccaccaacggggcgcagggggcgctggccgagcggctcaccgagaccacctgcatcgccgggccggctcccgccagccgagagcctcccgcgtcctcccccggggggacgcccttgacccagcgccgggaggactcggccctctga

SEQ ID NO: 3 - DNA, 1119 bp, Homo sapiens
atgttagccaacagctcctcaaccaacagttctgttctcccgtgtcctgactaccgacctacccaccgcctgcacttggtggtctacagcttggtgctggctgccgggctccccctcaacgcgctagccctctgggtcttcctgcgcgcgctgcgcgtgcactcggtggtgagcgtgtacatgtgtaacctggcggccagcgacctgctcttcaccctctcgctgcccgttcgtctctcctactacgcactgcaccactggcccttccccgacctcctgtgccagacgacgggcgccatcttccagatgaacatgtacggcagctgcatcttcctgatgctcatcaacgtggaccgctacgccgccatcgtgcacccgctgcgactgcgccacctgcggcggccccgcgtggcgcggctgctctgcctgggcgtgtgggcgctcatcctggtgtttgccgtgcccgccgcccgcgtgcacaggccctcgcgttgccgctaccgggacctcgaggtgcgcctatgcttcgagagcttcagcgacgagctgtggaaaggcaggctgctgcccctcgtgctgctggccgaggcgctgggcttcctgctgcccctggcggcggtggtctactcgtcgggccgagtcttctggacgctggcgcgccccgacgccacgcagagccagcggcggcggaagaccgtgcgcctcctgctggctaacctcgtcatcttcctgctgtgcttcgtgccctacaacagcacgctggcggtctacgggctgctgcggagcaagctggtggcggccagcgtgcctgcccgcgatcgcgtgcgcggggtgctgatggtgatggtgctgctggccggcgccaactgcgtgctggacccgctggtgtactactttagcgccgagggcttccgcaacaccctgcgcggcctgggcactccgcaccgggccaggacctcggccaccaacgggacgcgggcggcgctcgcgcaatccgaaaggtccgccgtcaccaccgacgccaccaggccggatgccgccagtcaggggctgctccgaccctccgactcccactctctgtcttccttcacacagtgtccccaggattccgccctctga

SEQ ID NO: 4 - protein, 373 aa, Felis catus
MLPNSTNSSVPPANGSVPPCPDYRPTHRLHMVAYSLVLAAGLPLNALALWVFLRALRVHSVVSVYMCNLAASDLLFTLSLPVRISYYALHYWPFSDLLCQTAGAIFQTNMYGSCIFLTLINVDRYAAIVHPLRLRHLRRPRVARLLCLGVWALILVFAVPTVLVHRPSSCSYGGGQVRLCFESFGDRLWKGGLLPLVLLAEALGFLLPLVAVLYSSGRVFWTLARPDATQSQRRRKTVRLLLANLVIFLLCFVPYNATLAVYGLLRGNLVAANSKVCDRVRGVLMVMVLLAGANCVLDPLVYYFSAEGFRNTLRGLGTPNRARTLATNGAQGALAEQPTETTYITTPATAEQGLLRPSNVGTPLTQLPEDSAL

SEQ ID NO: 5 - protein, 366 aa, Canis familiaris
MLTASANSSVPPCPDYRVTHRLHMVAYSLVLAAGLPLNALALWVFLRALRVHSVVSVYMCNLAASDLLFTLSLPVRISYYALHHWPFSDLLCQTAGAVFQTNMYGSCIFLTLINVDRYAAIVHPLRLRHLRRPRVARLLCLGVWALILVFAVPTVLVHRPSPCSYDGGRARLCFESFGDKLWKGGLLPLVLLAEALGFLLPLAAMLYSSGRVFWTLARPDATRSRRRRKTVRLLLANLVIFLLCFVPYNATLAVYGLLRGNLVAAGSEASDRVRQVLMVMVLLASANCVLDPLVYYFSAEGFRNTLRGLGTWHRARTLATNGAQGALAERLTETTCIAGPAPASREPPASSPGGTPLTQRREDSAL

SEQ ID NO: 6 - protein, 372 aa, Homo sapiens [sequence omitted]